European Patent Application EP 4 458 839 A1, published November 6, 2024. Title: Novel cell penetrating peptides and uses thereof. Applicant: 아주대학교 산학협력단. Application KR. The sequence listing filed with the application follows.

SEQUENCE LISTING (31 sequences)

SEQ ID NO: 1 - protein, 7 aa, synthetic construct
GCCGEIV

SEQ ID NO: 2 - protein, 7 aa, synthetic construct
ACCGEIV

SEQ ID NO: 3 - protein, 7 aa, synthetic construct
ICCGEIV

SEQ ID NO: 4 - protein, 7 aa, synthetic construct
LCCGEIV

SEQ ID NO: 5 - protein, 7 aa, synthetic construct
VCCGEIV

SEQ ID NO: 6 - protein, 7 aa, synthetic construct
NCCGEIV

SEQ ID NO: 7 - protein, 7 aa, synthetic construct
QCCGEIV

SEQ ID NO: 8 - protein, 7 aa, synthetic construct
RCCGEIV

SEQ ID NO: 9 - protein, 7 aa, synthetic construct
KCCGEIV

SEQ ID NO: 10 - protein, 7 aa, synthetic construct
DCCGEIV

SEQ ID NO: 11 - protein, 7 aa, synthetic construct
ECCGEIV

SEQ ID NO: 12 - protein, 7 aa, synthetic construct
YCCGEIV

SEQ ID NO: 13 - protein, 7 aa, synthetic construct
WCCGEIV

SEQ ID NO: 14 - protein, 7 aa, synthetic construct
FCCGEIV

SEQ ID NO: 15 - protein, 7 aa, synthetic construct
PCCGEIV

SEQ ID NO: 16 - protein, 7 aa, synthetic construct
GRCGEIV

SEQ ID NO: 17 - protein, 7 aa, synthetic construct
GCRGEIV

SEQ ID NO: 18 - protein, 7 aa, synthetic construct
GCCREIV

SEQ ID NO: 19 - protein, 7 aa, synthetic construct
GCCGRIV

SEQ ID NO: 20 - protein, 7 aa, synthetic construct
GCCGERV

SEQ ID NO: 21 - protein, 7 aa, synthetic construct
GCCGEIR

SEQ ID NO: 22 - protein, 15 aa, synthetic construct
GDDDDDDDDCCGEIV

SEQ ID NO: 23 - protein, 15 aa, synthetic construct
GCDDDDDDDDCGEIV

SEQ ID NO: 24 - protein, 15 aa, synthetic construct
GCCDDDDDDDDGEIV

SEQ ID NO: 25 - protein, 15 aa, synthetic construct
GCCGDDDDDDDDEIV

SEQ ID NO: 26 - protein, 15 aa, synthetic construct
GCCGEDDDDDDDDIV

SEQ ID NO: 27 - protein, 15 aa, synthetic construct
GCCGEIDDDDDDDDV

SEQ ID NO: 28 - protein, 15 aa, synthetic construct
GCCGEIVDDDDDDDD

SEQ ID NO: 29 - protein, 15 aa, synthetic construct
DDDDDDDDGCCGEIV

SEQ ID NO: 30 - protein, 23 aa, synthetic construct
DDDDDDDDGCCGEIVDDDDDDDD

SEQ ID NO: 31 - protein, 8 aa, synthetic construct
DDDDDDDD